European Patent Specification EP 3 704 243 B1, published August 30, 2023. Title: Modified Bacterial Spores. Applicant: Sporegen Limited. The sequence listing filed with the application follows.

SEQUENCE LISTING (19 sequences)

SEQ ID NO: 1 - DNA, 840 bp, Bacillus subtilis
atgacgcaattcgataaacaatacaattcaattataaaggatattatcaataatggaatctcagacgaagagtttgatgtaagaaccaagtgggactcagatggaacaccggcacatactctaagtgtaatcagtaagcaaatgagattcgacaactcagaggttccgattttaacgacaaaaaaggttgcctggaaaacagccattaaagagttgctctggatttggcagctgaaatctaatgatgttaatgatttaaacatgatgggcgtccatatttgggatcagtggaaacaagaagacggaaccatcggacatgcatatggatttcagctggggaagaaaaacagaagtctaaatggagaaaaagtggatcaggtagactatcttcttcatcaattgaagaacaatccatcttcacgcagacacattacaatgctgtggaatcctgatgaattagacgcaatggccttaacgccatgtgtatacgagacacaatggtacgttaaacatgggaaactccaccttgaggtaagagcacggagcaatgatatggcattgggaaatccattcaatgtattccagtataatgtgttgcagcgcatgattgctcaagtgactggttatgagcttggtgaatatatctttaacattggggattgccatgtgtacacacgtcatatagacaatttgaaaattcaaatggaaagagaacagtttgaagcacctgaactatggatcaatcctgaagtgaaagatttttatgactttaccattgatgatttcaagttaatcaactataaacatggggacaagcttttatttgaggtagcggtttaa

SEQ ID NO: 2 - DNA, 795 bp, Bacillus subtilis
atgaaacagtataaggatttctgcagacatgttttagagcatggtgagaaaaagggagaccggactgggaccggaacaatcagcactttcggatatcaaatgagatttaatttacgggaaggctttccgatgctcaccactaaaaaactccactttaaatcaattgcgcatgaactgctgtggttcttaaaaggagatacgaatgtacgctatctgcaggaaaacggagtgcgaatctggaatgagtgggctgatgaaaacggtgaacttggacctgtatatggctcccaatggcgttcttggcggggagctgatggagaaaccattgatcaaatttcccgtcttattgaagatattaaaacaaatccgaactccagacgcttaatcgtcagcgcctggaatgttggtgaaattgataaaatggcgttgccgccgtgccattgcctgttccaattctatgtgtctgacggcaagctgtcctgtcagctgtatcagcgctctgccgatgttttcttaggtgtgccgtttaatattgcatcttatgccctcctaaccatgatcattgctcatgtgactgggcttgaaccgggcgagttcatccatacgtttggtgatgttcatatttaccaaaatcatattgaacaagtcaatttgcagctggaaagagatgttagaccgcttccgcagcttcgtttcgccagaaaggttgattctatttttaactttgcatttgaggactttatcatcgaggattatgatccgcatcctcatataaaaggggcggtcagcgtatga

SEQ ID NO: 3 - DNA, 900 bp, Artificial Sequence
  left arm of thyA
cagatcatataaggaatgaaccgctgccaaatatcataaaaaagttgttaatgatcaaatgaatgaaattagagagaatttattttaaagaaagcccaattgcacatggacaaatgacaattgatattgaggtaaaatacaatgcattaaatcagaaaaagctattggaggatttaatgtgtttagacaatttccaatttggtatacacaaacacctgactatttgaatttttatgtaccgcaatatcaaaccatttcgtataatcctcaacaatgttatcaacggtgtatgtaccaaactggcggtaactatgagctatgtgacagactatgttatggagaaatacaggtgtaaaagagggggattaactcctctttaaacacacagtgagtggaataagatcctcactttatctgcaagtgcttagtatttgcgataatattgcattcgtaataaattatgcttagcaactgaaaatgaaagaaggatatgaatagtcatgacgcaattcgataaacaatacaattcaattataaaggatattatcaataatggaatctcagacgaagagtttgatgtaagaaccaagtgggactcagatggaacaccggcacatactctaagtgtaatcagtaagcaaatgagattcgacaactcagaggttccgattttaacgacaaaaaaggttgcctggaaaacagccattaaagagttgctctggatttggcagctgaaatctaatgatgttaatgatttaaacatgatgggcgtccatatttgggatcagtggaaacaagaagacggaaccatcggacatgcatatggatttcagctggggaagaaaaacagaagtctaaatggagaaaaagtggatcaggtagactatcttcttcatcaat

SEQ ID NO: 4 - DNA, 950 bp, Artificial Sequence
  right arm of thyA
tgaagaacaatccatcttcacgcagacacattacaatgctgtggaatcctgatgaattagacgcaatggccttaacgccatgtgtatacgagacacaatggtacgttaaacatgggaaactccaccttgaggtaagagcacggagcaatgatatggcattgggaaatccattcaatgtattccagtataatgtgttgcagcgcatgattgctcaagtgactggttatgagcttggtgaatatatctttaacattggggattgccatgtgtacacacgtcatatagacaatttgaaaattcaaatggaaagagaacagtttgaagcacctgaactatggatcaatcctgaagtgaaagatttttatgactttaccattgatgatttcaagttaatcaactataaacatggggacaagcttttatttgaggtagcggtttaatgctgcctttttattgtgcagtgaatagatagcaggtatcctaatttcattaagcaatctggaagatgaataaaaattgaaggacaaacacgtataatacataaaaaagattaactctacagttaatcttttttattcagaagaaaatatcctaactttgaaactaaatacaaagtaaaagcaatcattacagttctagatattacaattccatgaatagctagatcatatccagcaggtatcaacgcatttgtattacacataaaatatatagatattagaagtgctacaataactaaaatcattccaaaaagacttgttttttcatatttcataccaatttccacccttattaaagttaggtttaaacaaaagagctgaagaaacgaactatgaccagtatgctccaaggaaaaccgccagacaatgctggcggctttttgctgcttcgtttatttattaacagagatcgtaacgttatttcctgcaactgaaacctttgcgaaatcc

SEQ ID NO: 5 - DNA, 59 bp, Artificial Sequence
  multiple cloning site
agcttgcatgcctgcaggtcgactctagaggatcccccgggggtaccgagctcgaattc

SEQ ID NO: 6 - DNA, 1910 bp, Artificial Sequence
  thyA vector
cagatcatataaggaatgaaccgctgccaaatatcataaaaaagttgttaatgatcaaatgaatgaaattagagagaatttattttaaagaaagcccaattgcacatggacaaatgacaattgatattgaggtaaaatacaatgcattaaatcagaaaaagctattggaggatttaatgtgtttagacaatttccaatttggtatacacaaacacctgactatttgaatttttatgtaccgcaatatcaaaccatttcgtataatcctcaacaatgttatcaacggtgtatgtaccaaactggcggtaactatgagctatgtgacagactatgttatggagaaatacaggtgtaaaagagggggattaactcctctttaaacacacagtgagtggaataagatcctcactttatctgcaagtgcttagtatttgcgataatattgcattcgtaataaattatgcttagcaactgaaaatgaaagaaggatatgaatagtcatgacgcaattcgataaacaatacaattcaattataaaggatattatcaataatggaatctcagacgaagagtttgatgtaagaaccaagtgggactcagatggaacaccggcacatactctaagtgtaatcagtaagcaaatgagattcgacaactcagaggttccgattttaacgacaaaaaaggttgcctggaaaacagccattaaagagttgctctggatttggcagctgaaatctaatgatgttaatgatttaaacatgatgggcgtccatatttgggatcagtggaaacaagaagacggaaccatcggacatgcatatggatttcagctggggaagaaaaacagaagtctaaatggagaaaaagtggatcaggtagactatcttcttcatcaataagcttgcatgcctgcaggtcgactctagaggatcccccgggggtaccgagctcgaattctgaagaacaatccatcttcacgcagacacattacaatgctgtggaatcctgatgaattagacgcaatggccttaacgccatgtgtatacgagacacaatggtacgttaaacatgggaaactccaccttgaggtaagagcacggagcaatgatatggcattgggaaatccattcaatgtattccagtataatgtgttgcagcgcatgattgctcaagtgactggttatgagcttggtgaatatatctttaacattggggattgccatgtgtacacacgtcatatagacaatttgaaaattcaaatggaaagagaacagtttgaagcacctgaactatggatcaatcctgaagtgaaagatttttatgactttaccattgatgatttcaagttaatcaactataaacatggggacaagcttttatttgaggtagcggtttaatgctgcctttttattgtgcagtgaatagatagcaggtatcctaatttcattaagcaatctggaagatgaataaaaattgaaggacaaacacgtataatacataaaaaagattaactctacagttaatcttttttattcagaagaaaatatcctaactttgaaactaaatacaaagtaaaagcaatcattacagttctagatattacaattccatgaatagctagatcatatccagcaggtatcaacgcatttgtattacacataaaatatatagatattagaagtgctacaataactaaaatcattccaaaaagacttgttttttcatatttcataccaatttccacccttattaaagttaggtttaaacaaaagagctgaagaaacgaactatgaccagtatgctccaaggaaaaccgccagacaatgctggcggctttttgctgcttcgtttatttattaacagagatcgtaacgttatttcctgcaactgaaacctttgcgaaatcc

SEQ ID NO: 7 - DNA, 900 bp, Artificial Sequence
  left arm of thyB
ccaaatctgccgctcagtgtttgcatggagaatgtagaaaaagtcctgaacaaacgtgaaattattcatgctgttttgacaggccttgcactcgatcagcttgcagaacagaaacttctccccgaaccgctgcagcaccttgttgaaacggatgaaccgctttacggcatagatgaaattatcccgctttcaatcgttaatgtgtacgggtcgatcggtttgaccaatttcggttatttggataaagagaagattggaattattaaggaacttgatgaaagtccagacggtattcacacctttttggatgatattgtggcagctcttgctgcagcagcggcgagcagaattgcacatacgcatcaggatctgcaagatgaagaaaaagaacaggatgaaaagcctgtcgtcagctgactataaaaaaatcatttctgggttcagaaatgattttttattgtgttacactactagaagactacttttaaaggatgaaaaaaatgaaacagtataaggatttctgcagacatgttttagagcatggtgagaaaaagggagaccggactgggaccggaacaatcagcactttcggatatcaaatgagatttaatttacgggaaggctttccgatgctcaccactaaaaaactccactttaaatcaattgcgcatgaactgctgtggttcttaaaaggagatacgaatgtacgctatctgcaggaaaacggagtgcgaatctggaatgagtgggctgatgaaaacggtgaacttggacctgtatatggctcccaatggcgttcttggcggggagctgatggagaaaccattgatcaaatttcccgtcttattgaagatattaaaacaaatccgaactccagacgcttaatcgtcagcgcctgga

SEQ ID NO: 8 - DNA, 1095 bp, Artificial Sequence
  right arm of thyB
atgttggtgaaattgataaaatggcgttgccgccgtgccattgcctgttccaattctatgtgtctgacggcaagctgtcctgtcagctgtatcagcgctctgccgatgttttcttaggtgtgccgtttaatattgcatcttatgccctcctaaccatgatcattgctcatgtgactgggcttgaaccgggcgagttcatccatacgtttggtgatgttcatatttaccaaaatcatattgaacaagtcaatttgcagctggaaagagatgttagaccgcttccgcagcttcgtttcgccagaaaggttgattctatttttaactttgcatttgaggactttatcatcgaggattatgatccgcatcctcatataaaaggggcggtcagcgtatgatttcattcatttttgcgatggatgccaacaggcttatcggcaaagacaatgatttgccgtggcatttgcccaatgatcttgcatactttaagaaaataacatcgggccattcaatcattatgggccggaaaacatttgaatcgatcggacgtccgcttccaaatcggaaaaatattgtcgttacctcagcgccggattcagaatttcagggatgcacggttgtcagttcattaaaggatgtactggacatttgttcaggccctgaagaatgctttgtgatcggaggggctcagctctatacggacctgttcccttatgcggacagactgtatatgacgaaaattcatcacgagtttgagggtgaccgtcactttcctgaatttgatgaatccaattggaagctggtttcttctgagcaggggaccaaagacgaaaaaaacccgtatgattacgaatttctaatgtatgaaaaaaagaaatcttctaaagcgggaggattttaattggttcgctacagccttctagtggtttatattgtgtatatgctgttaaaaaatatgaaacaattatttaatcaaacaatgctcgatccccgtctgtcatacaaaaaacagatggctcttgtgtacgaacagccaaaggcgtttttagaaggctgtatcggcatctccggttcagttgtgacgatccatcagccaga

SEQ ID NO: 9 - DNA, 62 bp, Artificial Sequence
  multiple cloning site
aagcttgcatgcctgcaggtcgactctagaggatcccccgggggtaccgagctcgaattctg

SEQ ID NO: 10 - DNA, 2057 bp, Artificial Sequence
  thyB vector
ccaaatctgccgctcagtgtttgcatggagaatgtagaaaaagtcctgaacaaacgtgaaattattcatgctgttttgacaggccttgcactcgatcagcttgcagaacagaaacttctccccgaaccgctgcagcaccttgttgaaacggatgaaccgctttacggcatagatgaaattatcccgctttcaatcgttaatgtgtacgggtcgatcggtttgaccaatttcggttatttggataaagagaagattggaattattaaggaacttgatgaaagtccagacggtattcacacctttttggatgatattgtggcagctcttgctgcagcagcggcgagcagaattgcacatacgcatcaggatctgcaagatgaagaaaaagaacaggatgaaaagcctgtcgtcagctgactataaaaaaatcatttctgggttcagaaatgattttttattgtgttacactactagaagactacttttaaaggatgaaaaaaatgaaacagtataaggatttctgcagacatgttttagagcatggtgagaaaaagggagaccggactgggaccggaacaatcagcactttcggatatcaaatgagatttaatttacgggaaggctttccgatgctcaccactaaaaaactccactttaaatcaattgcgcatgaactgctgtggttcttaaaaggagatacgaatgtacgctatctgcaggaaaacggagtgcgaatctggaatgagtgggctgatgaaaacggtgaacttggacctgtatatggctcccaatggcgttcttggcggggagctgatggagaaaccattgatcaaatttcccgtcttattgaagatattaaaacaaatccgaactccagacgcttaatcgtcagcgcctggaaagcttgcatgcctgcaggtcgactctagaggatcccccgggggtaccgagctcgaattctgatgttggtgaaattgataaaatggcgttgccgccgtgccattgcctgttccaattctatgtgtctgacggcaagctgtcctgtcagctgtatcagcgctctgccgatgttttcttaggtgtgccgtttaatattgcatcttatgccctcctaaccatgatcattgctcatgtgactgggcttgaaccgggcgagttcatccatacgtttggtgatgttcatatttaccaaaatcatattgaacaagtcaatttgcagctggaaagagatgttagaccgcttccgcagcttcgtttcgccagaaaggttgattctatttttaactttgcatttgaggactttatcatcgaggattatgatccgcatcctcatataaaaggggcggtcagcgtatgatttcattcatttttgcgatggatgccaacaggcttatcggcaaagacaatgatttgccgtggcatttgcccaatgatcttgcatactttaagaaaataacatcgggccattcaatcattatgggccggaaaacatttgaatcgatcggacgtccgcttccaaatcggaaaaatattgtcgttacctcagcgccggattcagaatttcagggatgcacggttgtcagttcattaaaggatgtactggacatttgttcaggccctgaagaatgctttgtgatcggaggggctcagctctatacggacctgttcccttatgcggacagactgtatatgacgaaaattcatcacgagtttgagggtgaccgtcactttcctgaatttgatgaatccaattggaagctggtttcttctgagcaggggaccaaagacgaaaaaaacccgtatgattacgaatttctaatgtatgaaaaaaagaaatcttctaaagcgggaggattttaattggttcgctacagccttctagtggtttatattgtgtatatgctgttaaaaaatatgaaacaattatttaatcaaacaatgctcgatccccgtctgtcatacaaaaaacagatggctcttgtgtacgaacagccaaaggcgtttttagaaggctgtatcggcatctccggttcagttgtgacgatccatcagccaga

SEQ ID NO: 11 - protein, 272 aa, Artificial Sequence
  CotC-VP26
MGYYKKYKEEYYTVKKTYYKKYYEYDKKDYDCDYDKKYDDYDKKYYDHDKKDYDYVVEYKKHKKHYKLMEFGNLTNLDVAIIAILSIAIIALIVIMVIMIVFNTRVGRSVVANYDQMMRVPIQRRAKVMSIRGERSYNTPLGKVAMKNGLSDKDMKDVSADLVISTVTAPRTDPAGTGAENSNMTLKILNNTGVDLLINDITVRPTVIAGNIKGNTMSNTYFSSKDIKSSSSKITLIDVCSKFEDGAAFEATMNIGFTSKNVIDIKDEIKKK

SEQ ID NO: 12 - protein, 481 aa, Artificial Sequence
  CotB-VP28
MSKRRMKYHSNNEISYYNFLHSMKDKIVTVYRGGPESKKGKLTAVKSDYIALQAEKKIIYYQLEHVKSITEDTNNSTTTIETEEMLDADDFHSLIGHLINQSVQFNQGGPESKKGRLVWLGDDYAALNTNEDGVVYFNIHHIKSISKHEPDLKIEEQTPVGVLEADDLSEVFKSLTHKWVSINRGGPEAIEGILVDNADGHYTIVKNQEVLRIYPFHIKSISLGPKGSYKKEDQKNEQNQEDNNDKDSNSFISSKSYSSSKSSKRSLKSSDDQSSKLMDLSFTLSVVSAILAITAVIAVFIVIFRYHNTVTKTIETHTGNIETNMDENLRIPVTAEVGSGYFKMTDVSFDSDTLGKIKIRNGKSDAQMKEEDADLVITPVEGRALEVTVGQNLTFEGTFKVWNNTSRKINITGMQMVPKINPSKAFVGSSNTSSFTPVSIDEDEVGTFVCGTTFGAPIAATAGGNLFDMYVHVTYSGTETE

SEQ ID NO: 13 - protein, 597 aa, Artificial Sequence
  CotB-TcdA26-39
MSKRRMKYHSNNEISYYNFLHSMKDKIVTVYRGGPESKKGKLTAVKSDYIALQAEKKIIYYQLEHVKSITEDTNNSTTTIETEEMLDADDFHSLIGHLINQSVQFNQGGPESKKGRLVWLGDDYAALNTNEDGVVYFNIHHIKSISKHEPDLKIEEQTPVGVLEADDLSEVFKSLTHKWVSINRGGPEAIEGILVDNADGHYTIVKNQEVLRIYPFHIKSISLGPKGSYKKEDQKNEQNQEDNNDKDSNSFISSKSYSSSKSSKRSLKSSDDQSSKLASTGYTSINGKHFYFNTDGIMQIGVFKGPNGFEYFAPANTHNNNIEGQAILYQNKFLTLNGKKYYFGSDSKAVTGLRTIDGKKYYFNTNTAVAVTGWQTINGKKYYFNTNTSIASTGYTIISGKHFYFNTDGIMQIGVFKGPDGFEYFAPANTDANNIEGQAIRYQNRFLYLHDNIYYFGNNSKAATGWVTIDGNRYYFEPNTAMGANGYKTIDNKNFYFRNGLPQIGVFKGSNGFEYFAPANTDANNIEGQAIRYQNRFLHLLGKIYYFGNNSKAVTGWQTINGKVYYFMPDTAMAAAGGLFEIDGVIYFFGVDGVKAP

SEQ ID NO: 14 - protein, 388 aa, Artificial Sequence
  CotC-TcdA26-39
MGYYKKYKEEYYTVKKTYYKKYYEYDKKDYDCDYDKKYDDYDKKYYDHDKKDYDYVVEYKKHKKHYKLASTGYTSINGKHFYFNTDGIMQIGVFKGPNGFEYFAPANTHNNNIEGQAILYQNKFLTLNGKKYYFGSDSKAVTGLRTIDGKKYYFNTNTAVAVTGWQTINGKKYYFNTNTSIASTGYTIISGKHFYFNTDGIMQIGVFKGPDGFEYFAPANTDANNIEGQAIRYQNRFLYLHDNIYYFGNNSKAATGWVTIDGNRYYFEPNTAMGANGYKTIDNKNFYFRNGLPQIGVFKGSNGFEYFAPANTDANNIEGQAIRYQNRFLHLLGKIYYFGNNSKAVTGWQTINGKVYYFMPDTAMAAAGGLFEIDGVIYFFGVDGVKAP

SEQ ID NO: 15 - protein, 436 aa, Artificial Sequence
  CotB-SA
MSKRRMKYHSNNEISYYNFLHSMKDKIVTVYRGGPESKKGKLTAVKSDYIALQAEKKIIYYQLEHVKSITEDTNNSTTTIETEEMLDADDFHSLIGHLINQSVQFNQGGPESKKGRLVWLGDDYAALNTNEDGVVYFNIHHIKSISKHEPDLKIEEQTPVGVLEADDLSEVFKSLTHKWVSINRGGPEAIEGILVDNADGHYTIVKNQEVLRIYPFHIKSISLGPKGSYKKEDQKNEQNQEDNNDKDSNSFISSKSYSSSKSSKRSLKSSDDQSSIQDPSKDSKAQVSAAEAGITGTWYNQLGSTFIVTAGADGALTGTYESAVGNAESRYVLTGRYDSAPATDGSGTALGWTVAWKNNYRNAHSATTWSGQYVGGAEARINTQWLLTSGTTEANAWKSTLVGHDTFTKVKPSAASIDAAKKAGVNNGNPLDAVQQ

SEQ ID NO: 16 - protein, 552 aa, Artificial Sequence
  CotB-AprE
MSKRRMKYHSNNEISYYNFLHSMKDKIVTVYRGGPESKKGKLTAVKSDYIALQAEKKIIYYQLEHVKSITEDTNNSTTTIETEEMLDADDFHSLIGHLINQSVQFNQGGPESKKGRLVWLGDDYAALNTNEDGVVYFNIHHIKSISKHEPDLKIEEQTPVGVLEADDLSEVFKSLTHKWVSINRGGPEAIEGILVDNADGHYTIVKNQEVLRIYPFHIKSISLGPKGSYKKEDQKNEQNQEDNNDKDSNSFISSKSYSSSKSSKRSLKSSDDQSSKLAQSVPYGISQIKAPALHSQGYTGSNVKVAVIDSGIDSSHPDLNVRGGASFVPSETNPYQDGSSHGTHVAGTIAALNNSIGVLGVAPSASLYAVKVLDSTGSGQYSWIINGIEWAISNNMDVINMSLGGPTGSTALKTVVDKAVSSGIVVAAAAGNEGSSGSSSTVGYPAKYPSTIAVGAVNSSNQRASFSSAGSELDVMAPGVSIQSTLPGGTYGAYNGTSMATPHVAGAAALILSKHPTWTNAQVRDRLESTATYLGNSFYYGKGLINVQAAAQ

SEQ ID NO: 17 - protein, 903 aa, Artificial Sequence
  CotB-AmyE
MSKRRMKYHSNNEISYYNFLHSMKDKIVTVYRGGPESKKGKLTAVKSDYIALQAEKKIIYYQLEHVKSITEDTNNSTTTIETEEMLDADDFHSLIGHLINQSVQFNQGGPESKKGRLVWLGDDYAALNTNEDGVVYFNIHHIKSISKHEPDLKIEEQTPVGVLEADDLSEVFKSLTHKWVSINRGGPEAIEGILVDNADGHYTIVKNQEVLRIYPFHIKSISLGPKGSYKKEDQKNEQNQEDNNDKDSNSFISSKSYSSSKSSKRSLKSSDDQSSKLETANKSNEVAASSVKNGTILHAWNWSFNTLTQNMKEIRDAGYAAIQTSPINQVKEGNQGDKSMRNWYWLYQPTSYQIGNRYLGTEQEFKDMCAAAEKYGLKVIVDAVINHTTSDYAAISDEIKRIPNWTHGNTQIKNWSDRWDVTQNSLLGLYDWNTQNTEVQTYLKGFLERALNDGADGFRYDAAKHIELPDDGNYGSRFWPNITNTSAEFQYGEILQDSASRDTAYANYMNVTASNYGHSIRSALKNRNLSVSNISHYASDVSADKLVTWVESHDTYANDEEESTWMSDDDIRLGWAVIGSRSGSTPLFFSRPEGGGNGVRFPGKSQIGDRGSALFKDQAITAVNQFHNVMAGQPEELSNPNGNNQIFMNQRGSKGVVLANAGSSSVTVNTSTKLPDGRYDNRAGAGSFQVANGKLTGTINARSAAVLYSDDIGNAPQVFLENYQTGAVHSFNDQLTVTLRANAKTTKAVYQINNGQQTAFKDGDRLTIGKGDPIGTTYNIRLTGTNGEGAERTQEYTFVKKDPAQTNIIGYQNPDHWGQVNAYIYKHDGGGAIELTGSWPGKAMTKNANGIYTLTLPANADTANAKVIFNNGSAQVPGQNQPGFDYVQNGLYNNSGLNGYLPH

SEQ ID NO: 18 - protein, 279 aa, Artificial Sequence
  open reading frame of thyA
MTQFDKQYNSIIKDIINNGISDEEFDVRTKWDSDGTPAHTLSVISKQMRFDNSEVPILTTKKVAWKTAIKELLWIWQLKSNDVNDLNMMGVHIWDQWKQEDGTIGHAYGFQLGKKNRSLNGEKVDQVDYLLHQLKNNPSSRRHITMLWNPDELDAMALTPCVYETQWYVKHGKLHLEVRARSNDMALGNPFNVFQYNVLQRMIAQVTGYELGEYIFNIGDCHVYTRHIDNLKIQMEREQFEAPELWINPEVKDFYDFTIDDFKLINYKHGDKLLFEVAV

SEQ ID NO: 19 - protein, 264 aa, Artificial Sequence
  open reading frame of thyB
MKQYKDFCRHVLEHGEKKGDRTGTGTISTFGYQMRFNLREGFPMLTTKKLHFKSIAHELLWFLKGDTNVRYLQENGVRIWNEWADENGELGPVYGSQWRSWRGADGETIDQISRLIEDIKTNPNSRRLIVSAWNVGEIDKMALPPCHCLFQFYVSDGKLSCQLYQRSADVFLGVPFNIASYALLTMIIAHVTGLEPGEFIHTFGDVHIYQNHIEQVNLQLERDVRPLPQLRFARKVDSIFNFAFEDFIIEDYDPHPHIKGAVSV